European Patent Specification EP 3 574 109 B1, published July 26, 2023. Title: METHODS FOR CONSTRUCTING COPIES OF NUCLEIC ACID MOLECULES. Applicant: Tsavachidou, Dimitra. The sequence listing filed with the application follows.

SEQUENCE LISTING (1 sequence)

SEQ ID NO: 1 - DNA, 59 bp, Artificial Sequence
  Adaptor
ctcacacactttttttgagagagagagagagagagatttcctcagcttttgtgtgtgag